European Patent Specification EP 4 132 928 B1, published December 24, 2025. Title: INHIBITORS OF SARM1. Applicant: DISARM THERAPEUTICS, INC. The sequence listing filed with the application follows.

SEQUENCE LISTING (1 sequence)

SEQ ID NO: 1 - DNA, 6514 bp, Artificial Sequence
  Synthetic Construct
gcgatcgcggctcccgacatcttggaccattagctccacaggtatcttcttccctctagtggtcataacagcagcttcagctacctctcaattcaaaaaacccctcaagacccgtttagaggccccaaggggttatgctatcaatcgttgcgttacacacacaaaaaaccaacacacatccatcttcgatggatagcgattttattatctaactgctgatcgagtgtagccagatctagtaatcaattacggggtcattagttcatagcccatatatggagttccgcgttacataacttacggtaaatggcccgcctggctgaccgcccaacgacccccgcccattgacgtcaataatgacgtatgttcccatagtaacgccaatagggactttccattgacgtcaatgggtggagtatttacggtaaactgcccacttggcagtacatcaagtgtatcatatgccaagtacgccccctattgacgtcaatgacggtaaatggcccgcctggcattatgcccagtacatgaccttatgggactttcctacttggcagtacatctacgtattagtcatcgctattaccatgctgatgcggttttggcagtacatcaatgggcgtggatagcggtttgactcacggggatttccaagtctccaccccattgacgtcaatgggagtttgttttggcaccaaaatcaacgggactttccaaaatgtcgtaacaactccgccccattgacgcaaatgggcggtaggcgtgtacggtgggaggtctatataagcagagctggtttagtgaaccgtcagatcagatctttgtcgatcctaccatccactcgacacacccgccagcggccgctgccaagcttccgagctctcgaattcaaaggaggtacccaccatggccatgcatcaccaccaccatcatagctccggcgtcgacctcggcaccgagaatttatatttccaaagcggcctcaatgatatcttcgaggcccagaagatcgagtggcacgagggcagctccgacctcgccgtgcccggtcccgatggaggcggaggcactggtccttggtgggctgctggcggcagaggccctagagaagtgagccccggtgctggcaccgaggtgcaagacgctctggagagggctctgcccgaactgcagcaagctctgtccgctttaaagcaagctggaggagctagagccgtcggcgccggactggccgaagtgttccagctcgtggaggaagcttggttattacccgctgtgggaagagaggtcgcccaaggtctgtgtgacgccattcgtctggacggaggtttagacttattactgaggctgctgcaagctcccgaactggagacaagggtccaagctgctcgtctgctggagcagatcctcgtggccgagaatcgtgacagagtggctagaatcggtttaggcgtcatcctcaatttagccaaagagagggagcccgttgagctggccagaagcgtcgctggcatcctcgagcacatgttcaagcattccgaggagacttgtcagagactggtcgccgccggaggactcgatgctgttttatactggtgcagaaggacagaccccgctttactgaggcattgtgctctggccctcggcaattgcgctttacatggaggccaagccgtccagagaaggatggtggagaaaagagccgccgagtggctgttccctttagccttctccaaagaagacgaactgttacgtctgcatgcttgtctcgctgtcgctgttttagccaccaacaaggaggtggaaagggaagtggaaagaagcggaacactggctttagtcgaacctctggtggcttctttagatcccggaaggtttgccagatgtctggtcgacgccagcgatacctcccaaggaagaggccccgacgatctccagagactggtgcctctgctggacagcaatcgtctggaggcccaatgtattggcgccttctatctctgcgccgaagccgccatcaagtctttacaaggtaagaccaaggtgttctccgacattggagccatccaatctttaaagaggctggtgagctattccaccaacggcacaaaaagcgctttagccaaaagagctttaagactgctgggcgaagaggtgcctaggcccattttaccttccgtgcctagctggaaggaggccgaggtgcagacttggctgcagcagatcggctttagcaaatattgcgaatcctttagggagcagcaagttgacggcgatttattattaaggctgaccgaggaagagctccagacagatttaggcatgaaaagcggcatcactcgtaagaggttctttcgtgagctcaccgaactgaagaccttcgccaactactccacttgtgatcgtagcaatttagctgattggctcggatccctcgatcccagatttcgtcagtacacctatggactcgtctcttgtggactggacagatctttactgcatcgtgtgagcgagcaacagctgctggaagattgcggcatccatttaggagtgcacagagccagaattctgaccgccgctagagagatgctgcattcccctctcccttgtaccggaggcaagcctagcggagacacccccgacgtgttcatcagctatcgtagaaacagcggaagccagctggcctctttactgaaggtccatttacagctgcacggatttagcgtcttcatcgacgtggagaaactggaggctggcaagttcgaggacaagctgatccagtccgtgatgggcgctaggaatttcgttttagtgctcagccccggcgctctggataaatgcatgcaagatcatgactgtaaggactgggtccacaaggaaatcgtgaccgctctgtcttgtggcaagaacatcgtccccatcatcgacggcttcgaatggcccgagcctcaagttctccccgaagatatgcaagctgttttaaccttcaatggaatcaagtggagccacgagtaccaagaagccacaatcgagaagatcattcgttttctgcaaggtagatcctccagagattcctccgctggcagcgacacatctttagagggcgccgcccctatgggtcctacctaataatctagaagttgtctcctcctgcactgactgactgatacaatcgatttctggatccgcaggcctctgctagcttgactgactgagatacagcgtaccttcagctcacagacatgataagatacattgatgagtttggacaaaccacaactagaatgcagtgaaaaaaatgctttatttgtgaaatttgtgatgctattgctttatttgtaaccattataagctgcaataaacaagttaacaacaacaattgcattcattttatgtttcaggttcagggggaggtgtgggaggttttttaaagcaagtaaaacctctacaaatgtggtattggcccatctctatcggtatcgtagcataaccccttggggcctctaaacgggtcttgaggggttttttgtgcccctcgggccggattgctatctaccggcattggcgcagaaaaaaatgcctgatgcgacgctgcgcgtcttatactcccacatatgccagattcagcaacggatacggcttccccaacttgcccacttccatacgtgtcctccttaccagaaatttatccttaaggtcgtcagctatcctgcaggcgatctctcgatttcgatcaagacattcctttaatggtcttttctggacaccactaggggtcagaagtagttcatcaaactttcttccctccctaatctcattggttaccttgggctatcgaaacttaattaaccagtcaagtcagctacttggcgagatcgacttgtctgggtttcgactacgctcagaattgcgtcagtcaagttcgatctggtccttgctattgcacccgttctccgattacgagtttcatttaaatcatgtgagcaaaaggccagcaaaaggccaggaaccgtaaaaaggccgcgttgctggcgtttttccataggctccgcccccctgacgagcatcacaaaaatcgacgctcaagtcagaggtggcgaaacccgacaggactataaagataccaggcgtttccccctggaagctccctcgtgcgctctcctgttccgaccctgccgcttaccggatacctgtccgcctttctcccttcgggaagcgtggcgctttctcatagctcacgctgtaggtatctcagttcggtgtaggtcgttcgctccaagctgggctgtgtgcacgaaccccccgttcagcccgaccgctgcgccttatccggtaactatcgtcttgagtccaacccggtaagacacgacttatcgccactggcagcagccactggtaacaggattagcagagcgaggtatgtaggcggtgctacagagttcttgaagtggtggcctaactacggctacactagaagaacagtatttggtatctgcgctctgctgaagccagttaccttcggaaaaagagttggtagctcttgatccggcaaacaaaccaccgctggtagcggtggtttttttgtttgcaagcagcagattacgcgcagaaaaaaaggatctcaagaagatcctttgatcttttctacggggtctgacgctcagtggaacgaaaactcacgttaagggattttggtcatgagattatcaaaaaggatcttcacctagatccttttaaattaaaaatgaagttttaaatcaatctaaagtatatatgagtaaacttggtctgacagttaccaatgcttaatcagtgaggcacctatctcagcgatctgtctatttcgttcatccatagttgcatttaaatttccgaactctccaaggccctcgtcggaaaatcttcaaacctttcgtccgatccatcttgcaggctacctctcgaacgaactatcgcaagtctcttggccggccttgcgccttggctattgcttggcagcgcctatcgccaggtattactccaatcccgaatatccgagatcgggatcacccgagagaagttcaacctacatcctcaatcccgatctatccgagatccgaggaatatcgaaatcggggcgcgcctggtgtaccgagaacgatcctctcagtgcgagtctcgacgatccatatcgttgcttggcagtcagccagtcggaatccagcttgggacccaggaagtccaatcgtcagatattgtactcaagcctggtcacggcagcgtaccgatctgtttaaacctagatattgatagtctgatcggtcaacgtataatcgagtcctagcttttgcaaacatctatcaagagacaggatcagcaggaggctttcgcatgagtattcaacatttccgtgtcgcccttattcccttttttgcggcattttgccttcctgtttttgctcacccagaaacgctggtgaaagtaaaagatgctgaagatcagttgggtgcgcgagtgggttacatcgaactggatctcaacagcggtaagatccttgagagttttcgccccgaagaacgctttccaatgatgagcacttttaaagttctgctatgtggcgcggtattatcccgtattgacgccgggcaagagcaactcggtcgccgcatacactattctcagaatgacttggttgagtattcaccagtcacagaaaagcatcttacggatggcatgacagtaagagaattatgcagtgctgccataaccatgagtgataacactgcggccaacttacttctgacaacgattggaggaccgaaggagctaaccgcttttttgcacaacatgggggatcatgtaactcgccttgatcgttgggaaccggagctgaatgaagccataccaaacgacgagcgtgacaccacgatgcctgtagcaatggcaacaaccttgcgtaaactattaactggcgaactacttactctagcttcccggcaacagttgatagactggatggaggcggataaagttgcaggaccacttctgcgctcggcccttccggctggctggtttattgctgataaatctggagccggtgagcgtgggtctcgcggtatcattgcagcactggggccagatggtaagccctcccgtatcgtagttatctacacgacggggagtcaggcaactatggatgaacgaaatagacagatcgctgagataggtgcctcactgattaagcattggtaaccgattctaggtgcattggcgcagaaaaaaatgcctgatgcgacgctgcgcgtcttatactcccacatatgccagattcagcaacggatacggcttccccaacttgcccacttccatacgtgtcctccttaccagaaatttatccttaagatcccgaatcgtttaaactcgactctggctctatcgaatctccgtcgtttcgagcttacgcgaacagccgtggcgctcatttgctcgtcgggcatcgaatctcgtcagctatcgtcagcttacctttttggca